European Patent Specification EP 3 615 146 B1, published November 1, 2023. Title: HUMANIZED ANTIGEN-BINDING DOMAINS AND METHODS OF USE. Applicant: Kite Pharma, Inc. Wiltzius, Jed J.W. Sievers, Stuart A. The sequence listing filed with the application follows.

SEQUENCE LISTING (37 sequences)

SEQ ID NO: 1 - DNA, 816 bp, Artificial Sequence
  Synthetic Polynucleotide
atggaatggacctgggtgttcctgttcctgctgagcgtgacagccggcgtgcactctgacatccaaatgacgcaaacgacctcaagtctgtccgcgagcctgggcgaccgtgttacgattagctgccgtgcttcacaagatatcagtaaatacctgaactggtatcagcaaaaaccggatggtaccgttaaactgctgatctatcatacgtctcgtctgcacagtggcgtcccgtcccgctttagcggttctggcagtggtaccgattattcactgacgatttcgaacctggaacaggaagacatcgcgacctacttttgccagcaaggtaataccctgccgtatacgttcggcggtggcaccaaactggaaatcaccggctccacgtcaggctcgggtaaaccgggcagcggtgaaggctctaccaaaggtgaagtcaaactgcaggaaagcggtccgggtctggtcgcaccgagccaatctctgagtgtgacctgtacggtgtcgggtgttagcctgccggattacggcgtgtcatggattcgtcagccgccgcgtaaaggtctggaatggctgggtgttatctggggctcggaaaccacgtattacaatagtgcactgaaatcccgtctgaccattatcaaagacaactccaaatcacaggttttcctgaaaatgaacagcctgcaaaccgatgacacggcgatctattactgcgccaaacattattactatggtggctcttatgctatggattattggggtcaaggcacctcggttacggtctcgtcacatcatcatcatcatcattgataa

SEQ ID NO: 2 - DNA, 816 bp, Artificial Sequence
  Synthetic Polynucleotide
atggaatggacctgggtgttcctgttcctgctgagcgtgacagccggcgtgcactctgacatccaaatgacccagtcgccgtcctttctgagcgcaagcgtcggtgaccgtgttacgattacctgccgtgccagccaagacatctctaaatacctgaactggtatcagcaaaaaccggatcaggcaccgaaactgctgatcaaacatacctcacgtctgcactcgggtgtcccgagccgctttagtggttccggctcaggtaccgattttaccttcacgattagctctctgcagccggaagacatcgccacgtattactgccagcaaggtaataccctgccgtacacgttcggccaaggtaccaaactggaaatcaaaggctcgacgagcggctctggtaaaccgggctctggtgaaggcagtaccaaaggtgaagtgcagctggttgaaagcggtggtggtctggttcaaccgggtcgttccctgcgtctgtcatgtacggcgagtggtgtctccctgccggactatggcgtctcctgggtgcgtcagccgccgggtaaaggtctggaatggattggtgtgatctggggcagtgaaaccacgtattacaactcggccctgaaaagccgttttaccatttctcgcgataacagtaaaaatacgctgtacctgcagatgaatagcctgcgcgcggaagacaccgccgtttactactgcgcaaaacattactactacggtggcagctatgctatggactactggggtcagggcacgctggttacggtgtcgtcacatcatcatcatcatcattgataa

SEQ ID NO: 3 - DNA, 816 bp, Artificial Sequence
  Synthetic Polynucleotide
atggaatggacctgggtgttcctgttcctgctgagcgtgacagccggcgtgcactctgatattcaaatgacccagtccccgtcctccctgagtgcctccgtcggtgaccgtgttacgattacctgccgtgcgagccaagacatctctaaatacctgaactggtatcagcaaaaaccggatcaggcaccgaaactgctgatcaaacatacctcacgtctgcactcgggtgtgccgagccgctttagtggttccggctcaggtaccgattacaccctgacgatcagctctctgcagccggaagactttgccacgtattactgccagcaaggtaataccctgccgtatacgttcggccaaggtaccaaactggaaatcaaaggctcgacgagcggctctggtaaaccgggctctggtgaaggcagtaccaaaggtgaagtgcagctggttgaaagcggtggtggtctggttcaaccgggtcgttccctgcgtctgtcatgtacggcgagtggtgtctccctgccggactatggcgtgtcctggattcgtcagccgccgggtaaaggcctggaatggattggtgtcatctggggcagtgaaaccacgtattacaactcggccctgaaaagccgtttcaccatctctcgcgataacagtaaaaatacgctgtacctgcagatgaatagcctgcgcgcggaagacaccgccgtttactactgcgcaaaacattactactacggtggcagctatgctatggattactggggtcaaggcacgctggtcaccgtttcgtcacatcatcatcatcatcattgataa

SEQ ID NO: 4 - DNA, 650 bp, Artificial Sequence
  Synthetic Polynucleotide
atggaatggacctgggtgttcctgttcctgctgagcgtgacagccggcgtgcactctgacattcagatgacgcaaagtccgagtccggttcaggcaccgattttaccttcacgattagctctctgcaaccggaagacatcgccacgtattactgccagcaaggcaataccctgccgtacacgttcggtcagggcaccaaactggaaatcaaaggttcgacgagcggttctggcaaaccgggttctggcgaaggtagtaccaaaggccaggtccaactgcaggaaagcggcccgggtctggtgaaaccgtccggtaccctgtcactgacgtgtgcggtgagtggcgtttccctgccggactatggtgtttcctggattcgtcaaccgccgggcaaaggtctggaatggattggcgtcatctggggtagtgaaaccacgtattacaactcggccctgaaaagccgtgtgaccatctctcgcgataacagtaaaaatacgctgtacctgcagatgaatagcctgcgcgcggaagacaccgccgtttactactgcgcaaaacattactactacggcggtagctatgctatggattactggggtcaaggcacgctggttacggtttcctcgcatcatcatcatcatcactgataa

SEQ ID NO: 5 - DNA, 816 bp, Artificial Sequence
  Synthetic Polynucleotide
atggaatggacctgggtgttcctgttcctgctgagcgtgacagccggcgtgcactctgacattcagatgacacagagcccttcttccctgagcgccagcgtcggagatagagtgaccattacttgtagagccagccaggacatttccaaatacctgaactggtatcagcagaagcccgggaaagctgtgaagctgctgatctaccacacctctcggctgcatagtggagtcccttcaagattctcaggcagcgggtccggaactgactatactctgaccatcagctccctgcagcctgaggatattgcaacctacttctgccagcagggcaataccctgccatatacatttggcgggggaaccaaactggagattaaggggtctacaagtggctcagggaaaccaggaagcggcgaagggtccacaaagggccaggtgcagctgcaggagtctggaccaggcctggtgaagccctctgaaactctgagtgtcacatgtactgtgagcggagtctccctgcccgactacggcgtgagttggatcaggcagccccctgggaaaggactggagtggctgggcgtcatttgggggagcgaaaccacatactataactcagccctgaagagccggctgacaatctccaaagacacttctaagaatcaggtgtttctgaaaatgtctagtctgactgccgctgataccgcaatctactattgcgccaagcactactattacggcggctcctatgctatggattattgggggcaggggactctggtcactgtctcaagccatcatcatcatcatcattgataa

SEQ ID NO: 6 - protein, 19 aa, Artificial Sequence
  Synthetic Polypeptide
MEWTWVFLFLLSVTAGVHS

SEQ ID NO: 7 - protein, 18 aa, Artificial Sequence
  Synthetic Polypeptide
GSTSGSGKPGSGEGSTKG

SEQ ID NO: 8 - protein, 6 aa, Artificial Sequence
  Synthetic Polypeptide
HHHHHH

SEQ ID NO: 9 - protein, 270 aa, Artificial Sequence
  Synthetic Polypeptide
MEWTWVFLFLLSVTAGVHSDIQMTQTTSSLSASLGDRVTISCRASQDISKYLNWYQQKPDGTVKLLIYHTSRLHSGVPSRFSGSGSGTDYSLTISNLEQEDIATYFCQQGNTLPYTFGGGTKLEITGSTSGSGKPGSGEGSTKGEVKLQESGPGLVAPSQSLSVTCTVSGVSLPDYGVSWIRQPPRKGLEWLGVIWGSETTYYNSALKSRLTIIKDNSKSQVFLKMNSLQTDDTAIYYCAKHYYYGGSYAMDYWGQGTSVTVSSHHHHHH

SEQ ID NO: 10 - protein, 270 aa, Artificial Sequence
  Synthetic Polypeptide
MEWTWVFLFLLSVTAGVHSDIQMTQSPSFLSASVGDRVTITCRASQDISKYLNWYQQKPDQAPKLLIKHTSRLHSGVPSRFSGSGSGTDFTFTISSLQPEDIATYYCQQGNTLPYTFGQGTKLEIKGSTSGSGKPGSGEGSTKGEVQLVESGGGLVQPGRSLRLSCTASGVSLPDYGVSWVRQPPGKGLEWIGVIWGSETTYYNSALKSRFTISRDNSKNTLYLQMNSLRAEDTAVYYCAKHYYYGGSYAMDYWGQGTLVTVSSHHHHHH

SEQ ID NO: 11 - protein, 107 aa, Artificial Sequence
  Synthetic Polypeptide
DIQMTQSPSFLSASVGDRVTITCRASQDISKYLNWYQQKPDQAPKLLIKHTSRLHSGVPSRFSGSGSGTDFTFTISSLQPEDIATYYCQQGNTLPYTFGQGTKLEIK

SEQ ID NO: 12 - protein, 120 aa, Artificial Sequence
  Synthetic Polypeptide
EVQLVESGGGLVQPGRSLRLSCTASGVSLPDYGVSWVRQPPGKGLEWIGVIWGSETTYYNSALKSRFTISRDNSKNTLYLQMNSLRAEDTAVYYCAKHYYYGGSYAMDYWGQGTLVTVSS

SEQ ID NO: 13 - protein, 270 aa, Artificial Sequence
  Synthetic Polypeptide
MEWTWVFLFLLSVTAGVHSDIQMTQSPSSLSASVGDRVTITCRASQDISKYLNWYQQKPDQAPKLLIKHTSRLHSGVPSRFSGSGSGTDYTLTISSLQPEDFATYYCQQGNTLPYTFGQGTKLEIKGSTSGSGKPGSGEGSTKGEVQLVESGGGLVQPGRSLRLSCTASGVSLPDYGVSWIRQPPGKGLEWIGVIWGSETTYYNSALKSRFTISRDNSKNTLYLQMNSLRAEDTAVYYCAKHYYYGGSYAMDYWGQGTLVTVSSHHHHHH

SEQ ID NO: 14 - protein, 107 aa, Artificial Sequence
  Synthetic Polypeptide
DIQMTQSPSSLSASVGDRVTITCRASQDISKYLNWYQQKPDQAPKLLIKHTSRLHSGVPSRFSGSGSGTDYTLTISSLQPEDFATYYCQQGNTLPYTFGQGTKLEIK

SEQ ID NO: 15 - protein, 120 aa, Artificial Sequence
  Synthetic Polypeptide
EVQLVESGGGLVQPGRSLRLSCTASGVSLPDYGVSWIRQPPGKGLEWIGVIWGSETTYYNSALKSRFTISRDNSKNTLYLQMNSLRAEDTAVYYCAKHYYYGGSYAMDYWGQGTLVTVSS

SEQ ID NO: 16 - protein, 270 aa, Artificial Sequence
  Synthetic Polypeptide
MEWTWVFLFLLSVTAGVHSDIQMTQSPSTLSASVGDRVTITCRASQDISKYLNWYQQKPDQAPKLLIKHTSRLHSGVPSRFSGSGSGTDFTFTISSLQPEDIATYYCQQGNTLPYTFGQGTKLEIKGSTSGSGKPGSGEGSTKGQVQLQESGPGLVKPSGTLSLTCAVSGVSLPDYGVSWIRQPPGKGLEWIGVIWGSETTYYNSALKSRVTISRDNSKNTLYLQMNSLRAEDTAVYYCAKHYYYGGSYAMDYWGQGTLVTVSSHHHHHH

SEQ ID NO: 17 - protein, 107 aa, Artificial Sequence
  Synthetic Polypeptide
DIQMTQSPSTLSASVGDRVTITCRASQDISKYLNWYQQKPDQAPKLLIKHTSRLHSGVPSRFSGSGSGTDFTFTISSLQPEDIATYYCQQGNTLPYTFGQGTKLEIK

SEQ ID NO: 18 - protein, 120 aa, Artificial Sequence
  Synthetic Polypeptide
QVQLQESGPGLVKPSGTLSLTCAVSGVSLPDYGVSWIRQPPGKGLEWIGVIWGSETTYYNSALKSRVTISRDNSKNTLYLQMNSLRAEDTAVYYCAKHYYYGGSYAMDYWGQGTLVTVSS

SEQ ID NO: 19 - protein, 270 aa, Artificial Sequence
  Synthetic Polypeptide
MEWTWVFLFLLSVTAGVHSDIQMTQSPSSLSASVGDRVTITCRASQDISKYLNWYQQKPGKAVKLLIYHTSRLHSGVPSRFSGSGSGTDYTLTISSLQPEDIATYFCQQGNTLPYTFGGGTKLEIKGSTSGSGKPGSGEGSTKGQVQLQESGPGLVKPSETLSVTCTVSGVSLPDYGVSWIRQPPGKGLEWLGVIWGSETTYYNSALKSRLTISKDTSKNQVFLKMSSLTAADTAIYYCAKHYYYGGSYAMDYWGQGTLVTVSSHHHHHH

SEQ ID NO: 20 - protein, 107 aa, Artificial Sequence
  Synthetic Polypeptide
DIQMTQSPSSLSASVGDRVTITCRASQDISKYLNWYQQKPGKAVKLLIYHTSRLHSGVPSRFSGSGSGTDYTLTISSLQPEDIATYFCQQGNTLPYTFGGGTKLEIK

SEQ ID NO: 21 - protein, 120 aa, Artificial Sequence
  Synthetic Polypeptide
QVQLQESGPGLVKPSETLSVTCTVSGVSLPDYGVSWIRQPPGKGLEWLGVIWGSETTYYNSALKSRLTISKDTSKNQVFLKMSSLTAADTAIYYCAKHYYYGGSYAMDYWGQGTLVTVSS

SEQ ID NO: 22 - protein, 264 aa, Artificial Sequence
  Synthetic Polypeptide
MEWTWVFLFLLSVTAGVHSDIQMTQTTSSLSASLGDRVTISCRASQDISKYLNWYQQKPDGTVKLLIYHTSRLHSGVPSRFSGSGSGTDYSLTISNLEQEDIATYFCQQGNTLPYTFGGGTKLEITGSTSGSGKPGSGEGSTKGEVKLQESGPGLVAPSQSLSVTCTVSGVSLPDYGVSWIRQPPRKGLEWLGVIWGSETTYYNSALKSRLTIIKDNSKSQVFLKMNSLQTDDTAIYYCAKHYYYGGSYAMDYWGQGTSVTVSS

SEQ ID NO: 23 - protein, 264 aa, Artificial Sequence
  Synthetic Polypeptide
MEWTWVFLFLLSVTAGVHSDIQMTQSPSFLSASVGDRVTITCRASQDISKYLNWYQQKPDQAPKLLIKHTSRLHSGVPSRFSGSGSGTDFTFTISSLQPEDIATYYCQQGNTLPYTFGQGTKLEIKGSTSGSGKPGSGEGSTKGEVQLVESGGGLVQPGRSLRLSCTASGVSLPDYGVSWVRQPPGKGLEWIGVIWGSETTYYNSALKSRFTISRDNSKNTLYLQMNSLRAEDTAVYYCAKHYYYGGSYAMDYWGQGTLVTVSS

SEQ ID NO: 24 - protein, 264 aa, Artificial Sequence
  Synthetic Polypeptide
MEWTWVFLFLLSVTAGVHSDIQMTQSPSSLSASVGDRVTITCRASQDISKYLNWYQQKPDQAPKLLIKHTSRLHSGVPSRFSGSGSGTDYTLTISSLQPEDFATYYCQQGNTLPYTFGQGTKLEIKGSTSGSGKPGSGEGSTKGEVQLVESGGGLVQPGRSLRLSCTASGVSLPDYGVSWIRQPPGKGLEWIGVIWGSETTYYNSALKSRFTISRDNSKNTLYLQMNSLRAEDTAVYYCAKHYYYGGSYAMDYWGQGTLVTVSS

SEQ ID NO: 25 - protein, 264 aa, Artificial Sequence
  Synthetic Polypeptide
MEWTWVFLFLLSVTAGVHSDIQMTQSPSTLSASVGDRVTITCRASQDISKYLNWYQQKPDQAPKLLIKHTSRLHSGVPSRFSGSGSGTDFTFTISSLQPEDIATYYCQQGNTLPYTFGQGTKLEIKGSTSGSGKPGSGEGSTKGQVQLQESGPGLVKPSGTLSLTCAVSGVSLPDYGVSWIRQPPGKGLEWIGVIWGSETTYYNSALKSRVTISRDNSKNTLYLQMNSLRAEDTAVYYCAKHYYYGGSYAMDYWGQGTLVTVSS

SEQ ID NO: 26 - protein, 264 aa, Artificial Sequence
  Synthetic Polypeptide
MEWTWVFLFLLSVTAGVHSDIQMTQSPSSLSASVGDRVTITCRASQDISKYLNWYQQKPGKAVKLLIYHTSRLHSGVPSRFSGSGSGTDYTLTISSLQPEDIATYFCQQGNTLPYTFGGGTKLEIKGSTSGSGKPGSGEGSTKGQVQLQESGPGLVKPSETLSVTCTVSGVSLPDYGVSWIRQPPGKGLEWLGVIWGSETTYYNSALKSRLTISKDTSKNQVFLKMSSLTAADTAIYYCAKHYYYGGSYAMDYWGQGTLVTVSS

SEQ ID NO: 27 - protein, 11 aa, Artificial Sequence
  Synthetic Polypeptide
RASQDISKYLN

SEQ ID NO: 28 - protein, 7 aa, Artificial Sequence
  Synthetic Polypeptide
HTSRLHS

SEQ ID NO: 29 - protein, 9 aa, Artificial Sequence
  Synthetic Polypeptide
QQGNTLPYT

SEQ ID NO: 30 - protein, 7 aa, Artificial Sequence
  Synthetic Polypeptide
GVSLPDY

SEQ ID NO: 31 - protein, 5 aa, Artificial Sequence
  Synthetic Polypeptide
WGSET

SEQ ID NO: 32 - protein, 12 aa, Artificial Sequence
  Synthetic Polypeptide
HYYYGGSYAMDY

SEQ ID NO: 33 - protein, 5 aa, Artificial Sequence
  Synthetic Polypeptide
DYGVS

SEQ ID NO: 34 - protein, 16 aa, Artificial Sequence
  Synthetic Polypeptide
VIWGSETTYYNSALKS

SEQ ID NO: 35 - protein, 10 aa, Artificial Sequence
  Synthetic Polypeptide
GVSLPDYGVS

SEQ ID NO: 36 - protein, 107 aa, Artificial Sequence
  Synthetic Polypeptide
DIQMTQTTSSLSASLGDRVTISCRASQDISKYLNWYQQKPDGTVKLLIYHTSRLHSGVPSRFSGSGSGTDYSLTISNLEQEDIATYFCQQGNTLPYTFGGGTKLEIT

SEQ ID NO: 37 - protein, 120 aa, Artificial Sequence
  Synthetic Polypeptide
EVKLQESGPGLVAPSQSLSVTCTVSGVSLPDYGVSWIRQPPRKGLEWLGVIWGSETTYYNSALKSRLTIIKDNSKSQVFLKMNSLQTDDTAIYYCAKHYYYGGSYAMDYWGQGTSVTVSS